European Patent Application EP 4 549 451 A1, published May 7, 2025. Title: carrier peptide fragment and use thereof. Applicant: TOAGOSEI CO., LTD. The sequence listing filed with the application follows.

SEQUENCE LISTING (5 sequences)

SEQ ID NO: 1 - protein, 14 aa, synthetic construct
KKRTLRKSNSRKKR

SEQ ID NO: 2 - protein, 14 aa, synthetic construct
KKRTLRKSSNRKKR

SEQ ID NO: 3 - protein, 14 aa, synthetic construct
KKRTLRKSNNRKKR

SEQ ID NO: 4 - protein, 14 aa, synthetic construct
KKRTLRKNSNRKKR

SEQ ID NO: 5 - protein, 14 aa, synthetic construct
VVRSLVKVVRSLVK